European Patent Application EP 4 289 964 A1, published December 13, 2023. Title: PRIMER-PROBE COMBINATION AND KIT FOR VAGINAL MICROECOSYSTEM DETECTION. Applicant: BEIJING ORIGINPOLY BIO-TEC CO., LTD. The sequence listing filed with the application follows.

SEQUENCE LISTING (32 sequences)

SEQ ID NO: 1 - DNA, 24 bp, synthetic construct
  source 1..24: mol_type = other DNA
  modified_base 8: mod_base = OTHER; note = Locked nucleic acid thymine
  modified_base 9: mod_base = OTHER; note = Locked nucleic acid adenosine
  modified_base 10: mod_base = OTHER; note = Locked nucleic acid adenosine
  modified_base 11: mod_base = OTHER; note = Locked nucleic acid thymine
ctttcggtaatgacgttaggaaag

SEQ ID NO: 2 - DNA, 23 bp, synthetic construct
  source 1..23: mol_type = other DNA
  modified_base 10: mod_base = OTHER; note = Locked nucleic acid thymine
  modified_base 11: mod_base = OTHER; note = Locked nucleic acid cytosine
  modified_base 12: mod_base = OTHER; note = Locked nucleic acid thymine
  modified_base 13: mod_base = OTHER; note = Locked nucleic acid thymine
aatacgctttcttatccggtatt

SEQ ID NO: 3 - DNA, 18 bp, synthetic construct
  source 1..18: mol_type = other DNA
  modified_base 1: mod_base = OTHER; note = Carboxyfluorescein cytosine
  modified_base 3: mod_base = OTHER; note = Locked nucleic acid guanosine
  modified_base 11: mod_base = OTHER; note = Locked nucleic acid guanosine
  modified_base 18: mod_base = OTHER; note = Adenosine minor groove binder
cggcggatgggtgagtaa

SEQ ID NO: 4 - DNA, 19 bp, synthetic construct
  source 1..19: mol_type = other DNA
  modified_base 5: mod_base = OTHER; note = Locked nucleic acid thymine
  modified_base 7: mod_base = OTHER; note = Locked nucleic acid adenosine
  modified_base 8: mod_base = OTHER; note = Locked nucleic acid cytosine
  modified_base 10: mod_base = OTHER; note = Locked nucleic acid thymine
gtgttgacctgggctacac

SEQ ID NO: 5 - DNA, 19 bp, synthetic construct
  source 1..19: mol_type = other DNA
  modified_base 5: mod_base = OTHER; note = Locked nucleic acid cytosine
  modified_base 12: mod_base = OTHER; note = Locked nucleic acid cytosine
ccttccagcttcgtgtagg

SEQ ID NO: 6 - DNA, 16 bp, synthetic construct
  source 1..16: mol_type = other DNA
  modified_base 1: mod_base = OTHER; note = Carboxyfluorescein thymine
  modified_base 4: mod_base = OTHER; note = Locked nucleic acid adenosine
  modified_base 7: mod_base = OTHER; note = Locked nucleic acid guanosine
  modified_base 10: mod_base = OTHER; note = Locked nucleic acid cytosine
  modified_base 16: mod_base = OTHER; note = Guanosine minor groove binder
tggacggtacaacgag

SEQ ID NO: 7 - DNA, 26 bp, synthetic construct
  source 1..26: mol_type = other DNA
  modified_base 14: mod_base = OTHER; note = Locked nucleic acid adenosine
  modified_base 15: mod_base = OTHER; note = Locked nucleic acid guanosine
gaaaccacctaagagattaggttttc

SEQ ID NO: 8 - DNA, 24 bp, synthetic construct
  source 1..24: mol_type = other DNA
  modified_base 10: mod_base = OTHER; note = Locked nucleic acid cytosine
cagcgagtgcccaacttaatgctg

SEQ ID NO: 9 - DNA, 21 bp, synthetic construct
  source 1..21: mol_type = other DNA
  modified_base 1: mod_base = OTHER; note = Carboxyfluorescein cytosine
  modified_base 3: mod_base = OTHER; note = Locked nucleic acid guanosine
  modified_base 4: mod_base = OTHER; note = Locked nucleic acid guanosine
  modified_base 6: mod_base = OTHER; note = Locked nucleic acid adenosine
  modified_base 9: mod_base = OTHER; note = Locked nucleic acid adenosine
  modified_base 10: mod_base = OTHER; note = Locked nucleic acid adenosine
  modified_base 21: mod_base = OTHER; note = Guanosine minor groove binder
cggggacaaagagacaggtgg

SEQ ID NO: 10 - DNA, 21 bp, synthetic construct
  source 1..21: mol_type = other DNA
  modified_base 9: mod_base = OTHER; note = Locked nucleic acid guanosine
  modified_base 12: mod_base = OTHER; note = Locked nucleic acid thymine
ccctgcgtgagtgaagaaggg

SEQ ID NO: 11 - DNA, 19 bp, synthetic construct
  source 1..19: mol_type = other DNA
  modified_base 9: mod_base = OTHER; note = Locked nucleic acid adenosine
  modified_base 11: mod_base = OTHER; note = Locked nucleic acid cytosine
gcagtattaccgcggctgc

SEQ ID NO: 12 - DNA, 21 bp, synthetic construct
  source 1..21: mol_type = other DNA
  modified_base 1: mod_base = OTHER; note = Carboxyfluorescein guanosine
  modified_base 5: mod_base = OTHER; note = Locked nucleic acid thymine
  modified_base 7: mod_base = OTHER; note = Locked nucleic acid thymine
  modified_base 8: mod_base = OTHER; note = Locked nucleic acid thymine
  modified_base 10: mod_base = OTHER; note = Locked nucleic acid thymine
  modified_base 11: mod_base = OTHER; note = Locked nucleic acid thymine
  modified_base 12: mod_base = OTHER; note = Locked nucleic acid guanosine
  modified_base 21: mod_base = OTHER; note = Guanosine minor groove binder
gctctgttgttggtgaagaag

SEQ ID NO: 13 - DNA, 21 bp, synthetic construct
  source 1..21: mol_type = other DNA
  modified_base 8: mod_base = OTHER; note = Locked nucleic acid thymine
  modified_base 10: mod_base = OTHER; note = Locked nucleic acid guanosine
gccacggttggtgagagtggc

SEQ ID NO: 14 - DNA, 19 bp, synthetic construct
  source 1..19: mol_type = other DNA
  modified_base 10: mod_base = OTHER; note = Locked nucleic acid adenosine
  modified_base 11: mod_base = OTHER; note = Locked nucleic acid guanosine
  modified_base 12: mod_base = OTHER; note = Locked nucleic acid thymine
  modified_base 13: mod_base = OTHER; note = Locked nucleic acid thymine
tgctcgtcaagttggagca

SEQ ID NO: 15 - DNA, 14 bp, synthetic construct
  source 1..14: mol_type = other DNA
  modified_base 1: mod_base = OTHER; note = Carboxyfluorescein thymine
  modified_base 4: mod_base = OTHER; note = Locked nucleic acid guanosine
  modified_base 14: mod_base = OTHER; note = Thymine minor groove binder
tgcgtgaccaacct

SEQ ID NO: 16 - DNA, 19 bp, synthetic construct
  source 1..19: mol_type = other DNA
  modified_base 8: mod_base = OTHER; note = Locked nucleic acid guanosine
  modified_base 11: mod_base = OTHER; note = Locked nucleic acid adenosine
ccgctaggtgaacctgcgg

SEQ ID NO: 17 - DNA, 21 bp, synthetic construct
  source 1..21: mol_type = other DNA
  modified_base 6: mod_base = OTHER; note = Locked nucleic acid adenosine
  modified_base 9: mod_base = OTHER; note = Locked nucleic acid guanosine
  modified_base 11: mod_base = OTHER; note = Locked nucleic acid adenosine
gaaccaaagcaagtttgtttc

SEQ ID NO: 18 - DNA, 11 bp, synthetic construct
  source 1..11: mol_type = other DNA
  modified_base 1: mod_base = OTHER; note = Carboxyfluorescein Locked nucleic acid adenosine
  modified_base 3: mod_base = OTHER; note = Locked nucleic acid thymine
  modified_base 4: mod_base = OTHER; note = Locked nucleic acid guanosine
  modified_base 5: mod_base = OTHER; note = Locked nucleic acid adenosine
  modified_base 8: mod_base = OTHER; note = Locked nucleic acid thymine
  modified_base 11: mod_base = OTHER; note = Thymine minor groove binder
actgatttggt

SEQ ID NO: 19 - DNA, 20 bp, synthetic construct
  source 1..20: mol_type = other DNA
  modified_base 5: mod_base = OTHER; note = Locked nucleic acid guanosine
  modified_base 6: mod_base = OTHER; note = Locked nucleic acid cytosine
gagggccacatgaatgactc

SEQ ID NO: 20 - DNA, 21 bp, synthetic construct
  source 1..21: mol_type = other DNA
  modified_base 6: mod_base = OTHER; note = Locked nucleic acid guanosine
  modified_base 8: mod_base = OTHER; note = Locked nucleic acid guanosine
  modified_base 11: mod_base = OTHER; note = Locked nucleic acid adenosine
ggggtgagatagatctacccc

SEQ ID NO: 21 - DNA, 14 bp, synthetic construct
  source 1..14: mol_type = other DNA
  modified_base 1: mod_base = OTHER; note = Carboxyfluorescein cytosine
  modified_base 2: mod_base = OTHER; note = Locked nucleic acid adenosine
  modified_base 4: mod_base = OTHER; note = Locked nucleic acid thymine
  modified_base 6: mod_base = OTHER; note = Locked nucleic acid thymine
  modified_base 8: mod_base = OTHER; note = Locked nucleic acid adenosine
  modified_base 11: mod_base = OTHER; note = Locked nucleic acid thymine
  modified_base 14: mod_base = OTHER; note = Thymine minor groove binder
cagtatgaagtctt

SEQ ID NO: 22 - DNA, 19 bp, synthetic construct
  source 1..19: mol_type = other DNA
aagggtgcagctgagctag

SEQ ID NO: 23 - DNA, 19 bp, synthetic construct
  source 1..19: mol_type = other DNA
gcacaagctttgtacatgg

SEQ ID NO: 24 - DNA, 22 bp, synthetic construct
  source 1..22: mol_type = other DNA
  modified_base 1: mod_base = OTHER; note = Hexane cytosine
  modified_base 22: mod_base = OTHER; note = Cytosine Black hole quencher-1
cagcaagcattcctggggtggc

SEQ ID NO: 25 - DNA, 110 bp, Lactobacillus crispatus
  source 1..110: mol_type = unassigned DNA
ggtaatgacgttaggaaagcgagcggcggatgggtgagtaacacgtggggaacctgccccatagtctgggataccacttggaaacaggtgctaataccggataagaaagc

SEQ ID NO: 26 - DNA, 126 bp, Lactobacillus gasseri
  source 1..126: mol_type = unassigned DNA
tgacctgggctacacacgtgctacaatggacggtacaacgagaagcgaacctgcgaaggcaagcggatctctgaaagccgttctcagttcggactgtaggctgcaactcgcctacacgaagctgga

SEQ ID NO: 27 - DNA, 144 bp, Lactobacillus jensenii
  source 1..144: mol_type = unassigned DNA
ccacctaagagattaggttttcccttcggggacaaagagacaggtggtgcatggctgtcgtcagctcgtgtcgtgagatgttgggttaagtcccgcaacgagcgcaacccttgttaatagttgccagcattaagttgggcactc

SEQ ID NO: 28 - DNA, 135 bp, Lactobacillus iners
  source 1..135: mol_type = unassigned DNA
gcgtgagtgaagaagggtttcggctcgtaaagctctgttgttggtgaagaaggacaggggtagtaactgacctttgtttgacggtaatcaattagaaagtcacggctaactacgtgccagcagccgcggtaatac

SEQ ID NO: 29 - DNA, 105 bp, Gardnerella vaginalis
  source 1..105: mol_type = unassigned DNA
ggttggtgagagtggcgaacgggtgagtaatgcgtgaccaacctgccccatgctccagaatagctcttggaaacgggtggtaatgctggatgctccaacttgacg

SEQ ID NO: 30 - DNA, 80 bp, Candida albicans
  source 1..80: mol_type = unassigned DNA
taggtgaacctgcggaaggatcattactgatttggtgaattgcaccacatgtgtttttctttgaaacaaacttgctttgg

SEQ ID NO: 31 - DNA, 89 bp, Trichomonas vaginalis
  source 1..89: mol_type = unassigned DNA
ggccacatgaatgactcagcgcagtatgaagtctttgttttcttccgaaaacaagctcaatgagagccatcgggggtagatctatctca

SEQ ID NO: 32 - DNA, 82 bp, synthetic construct
  source 1..82: mol_type = other DNA
aagggtgcagctgagctaggcagcagcaagcattcctggggtggcatagtggggtggtgaataccatgtacaaagcttgtgc